European Patent Specification EP 3 685 847 B1, published January 11, 2023. Title: MODULATORS OF COMPLEMENT ACTIVITY. Applicant: RA PHARMACEUTICALS, INC. Application EP 16823378.1. The sequence listing filed with the application follows.

SEQUENCE LISTING (1 sequence)

SEQ ID NO: 1 - protein, 15 aa, Artificial Sequence
  Description of Artificial Sequence: Synthetic peptide
  N-term Ac
  MOD_RES (1)..(6): Lactam bridge between residues
  MOD_RES (7)..(7): (N-Me)Asp
  MOD_RES (8)..(8): Tert-butyl-Gly
  MOD_RES (10)..(10): 7-aza-Trp
  MOD_RES (14)..(14): Cyclohexyl-Gly
  MOD_RES (15)..(15): N-epsilon-(PEG24-gamma-glutamic acid-N-alpha- hexadecanoyl)Lys
KVERFDDGYWEYPGK